European Patent Application EP 4 660 204 A1, published December 10, 2025. Title: ANTAGONIST FOR USE IN TREATMENT OF MEMBRANOUS NEPHROPATHY. Applicant: Chang Gung University. Application TW. The sequence listing filed with the application follows.

SEQUENCE LISTING (191 sequences)

SEQ ID NO: 1 - DNA, 20 bp, synthetic construct
  source 1..20: mol_type = other DNA
accatggactgsacctggag

SEQ ID NO: 2 - DNA, 24 bp, synthetic construct
  source 1..24: mol_type = other DNA
caccatggacacactttgctmcac

SEQ ID NO: 3 - DNA, 24 bp, synthetic construct
  source 1..24: mol_type = other DNA
accatggacatactttgttccacg

SEQ ID NO: 4 - DNA, 20 bp, synthetic construct
  source 1..20: mol_type = other DNA
atggagtttgggctgagctg

SEQ ID NO: 5 - DNA, 20 bp, synthetic construct
  source 1..20: mol_type = other DNA
atggaactggggctccgctg

SEQ ID NO: 6 - DNA, 20 bp, synthetic construct
  source 1..20: mol_type = other DNA
atggagttggggctgtgctg

SEQ ID NO: 7 - DNA, 21 bp, synthetic construct
  source 1..21: mol_type = other DNA
catggagtttgggcttagctg

SEQ ID NO: 8 - DNA, 21 bp, synthetic construct
  source 1..21: mol_type = other DNA
catggagttttggctgagctg

SEQ ID NO: 9 - DNA, 24 bp, synthetic construct
  source 1..24: mol_type = other DNA
catgaaacacctgtggttcttcct

SEQ ID NO: 10 - DNA, 24 bp, synthetic construct
  source 1..24: mol_type = other DNA
aatgaagcacctgtggttcttcct

SEQ ID NO: 11 - DNA, 25 bp, synthetic construct
  source 1..25: mol_type = other DNA
acatgaaacatctgtggttcttcct

SEQ ID NO: 12 - DNA, 20 bp, synthetic construct
  source 1..20: mol_type = other DNA
atggggtcaaccgccatcct

SEQ ID NO: 13 - DNA, 27 bp, synthetic construct
  source 1..27: mol_type = other DNA
aatgtctgtctccttcctcatcttcct

SEQ ID NO: 14 - DNA, 20 bp, synthetic construct
  source 1..20: mol_type = other DNA
saggtgcagctggtgsagtc

SEQ ID NO: 15 - DNA, 20 bp, synthetic construct
  source 1..20: mol_type = other DNA
caggtccagcttgtgcagtc

SEQ ID NO: 16 - DNA, 20 bp, synthetic construct
  source 1..20: mol_type = other DNA
caggttcagctggtgcagtc

SEQ ID NO: 17 - DNA, 22 bp, synthetic construct
  source 1..22: mol_type = other DNA
caggtccagctggtacagtctg

SEQ ID NO: 18 - DNA, 23 bp, synthetic construct
  source 1..23: mol_type = other DNA
caggtcacctgarggagtctggt

SEQ ID NO: 19 - DNA, 21 bp, synthetic construct
  source 1..21: mol_type = other DNA
gaggtgcagctgttggagtct

SEQ ID NO: 20 - DNA, 19 bp, synthetic construct
  source 1..19: mol_type = other DNA
cagstgcagctgcaggagt

SEQ ID NO: 21 - DNA, 21 bp, synthetic construct
  source 1..21: mol_type = other DNA
caggtgcagctacarcagtgg

SEQ ID NO: 22 - DNA, 21 bp, synthetic construct
  source 1..21: mol_type = other DNA
caggtacagctgcagcagtca

SEQ ID NO: 23 - DNA, 19 bp, synthetic construct
  source 1..19: mol_type = other DNA
caggtgcagctggtgcaat

SEQ ID NO: 24 - DNA, 20 bp, synthetic construct
  source 1..20: mol_type = other DNA
ggtccccgctcagctcctgg

SEQ ID NO: 25 - DNA, 20 bp, synthetic construct
  source 1..20: mol_type = other DNA
agtcctcgctcagctcctgg

SEQ ID NO: 26 - DNA, 20 bp, synthetic construct
  source 1..20: mol_type = other DNA
gctccctgctcagctcctgg

SEQ ID NO: 27 - DNA, 20 bp, synthetic construct
  source 1..20: mol_type = other DNA
gctccttgctcagcttctgg

SEQ ID NO: 28 - DNA, 20 bp, synthetic construct
  source 1..20: mol_type = other DNA
cctgctactctggctcccag

SEQ ID NO: 29 - DNA, 25 bp, synthetic construct
  source 1..25: mol_type = other DNA
atttctctgttgctctggatctctg

SEQ ID NO: 30 - DNA, 23 bp, synthetic construct
  source 1..23: mol_type = other DNA
cttcctcctcctttggatctctg

SEQ ID NO: 31 - DNA, 20 bp, synthetic construct
  source 1..20: mol_type = other DNA
tctgctgctctgggttccag

SEQ ID NO: 32 - DNA, 23 bp, synthetic construct
  source 1..23: mol_type = other DNA
gacatccagwtgacccagtctcc

SEQ ID NO: 33 - DNA, 28 bp, synthetic construct
  source 1..28: mol_type = other DNA
gatattgtgatgacccagactccactct

SEQ ID NO: 34 - DNA, 28 bp, synthetic construct
  source 1..28: mol_type = other DNA
gatattgtgatgactcagtctccactct

SEQ ID NO: 35 - DNA, 25 bp, synthetic construct
  source 1..25: mol_type = other DNA
gaaattgtgttgacrcagtctccag

SEQ ID NO: 36 - DNA, 25 bp, synthetic construct
  source 1..25: mol_type = other DNA
gaaatagtgatgacgcagtctccag

SEQ ID NO: 37 - DNA, 22 bp, synthetic construct
  source 1..22: mol_type = other DNA
gacatcgtgatgacccagtctc

SEQ ID NO: 38 - DNA, 22 bp, synthetic construct
  source 1..22: mol_type = other DNA
gaaacgacactcacgcagtctc

SEQ ID NO: 39 - DNA, 24 bp, synthetic construct
  source 1..24: mol_type = other DNA
gaaattgtgctgactcagtctcca

SEQ ID NO: 40 - DNA, 20 bp, synthetic construct
  source 1..20: mol_type = other DNA
ggtcctgggcccagtctgtg

SEQ ID NO: 41 - DNA, 20 bp, synthetic construct
  source 1..20: mol_type = other DNA
ggtcctgggcycagtctgcc

SEQ ID NO: 42 - DNA, 22 bp, synthetic construct
  source 1..22: mol_type = other DNA
gctctgwggcctcctatgagct

SEQ ID NO: 43 - DNA, 23 bp, synthetic construct
  source 1..23: mol_type = other DNA
gctctgtgacctcctatgwgctg

SEQ ID NO: 44 - DNA, 26 bp, synthetic construct
  source 1..26: mol_type = other DNA
gttctgtggtttcttctgagctgact

SEQ ID NO: 45 - DNA, 21 bp, synthetic construct
  source 1..21: mol_type = other DNA
ggtctctctcccwgcytgtgc

SEQ ID NO: 46 - DNA, 20 bp, synthetic construct
  source 1..20: mol_type = other DNA
gttccctctcgcaggctgtg

SEQ ID NO: 47 - DNA, 20 bp, synthetic construct
  source 1..20: mol_type = other DNA
gktccctctcccagcctgtg

SEQ ID NO: 48 - DNA, 23 bp, synthetic construct
  source 1..23: mol_type = other DNA
gttcttgggccaattttatgctg

SEQ ID NO: 49 - DNA, 23 bp, synthetic construct
  source 1..23: mol_type = other DNA
ggtccaattcycagrctgtggtg

SEQ ID NO: 50 - DNA, 24 bp, synthetic construct
  source 1..24: mol_type = other DNA
gagtggattctcagactgtggtga

SEQ ID NO: 51 - DNA, 20 bp, synthetic construct
  source 1..20: mol_type = other DNA
tgtcagtggtccaggcaggg

SEQ ID NO: 52 - DNA, 20 bp, synthetic construct
  source 1..20: mol_type = other DNA
cagtctgtgytgacgcagcc

SEQ ID NO: 53 - DNA, 21 bp, synthetic construct
  source 1..21: mol_type = other DNA
cagtctgtgctgactcagcca

SEQ ID NO: 54 - DNA, 20 bp, synthetic construct
  source 1..20: mol_type = other DNA
cagtctgccctgactcagcc

SEQ ID NO: 55 - DNA, 21 bp, synthetic construct
  source 1..21: mol_type = other DNA
tcctatgagctgacwcagcca

SEQ ID NO: 56 - DNA, 22 bp, synthetic construct
  source 1..22: mol_type = other DNA
tcttctgagctgactcaggacc

SEQ ID NO: 57 - DNA, 20 bp, synthetic construct
  source 1..20: mol_type = other DNA
cagsctgtgctgactcagcc

SEQ ID NO: 58 - DNA, 22 bp, synthetic construct
  source 1..22: mol_type = other DNA
cagcctgtgctgactcaatcat

SEQ ID NO: 59 - DNA, 21 bp, synthetic construct
  source 1..21: mol_type = other DNA
cagcttgtgctgactcaatcg

SEQ ID NO: 60 - DNA, 24 bp, synthetic construct
  source 1..24: mol_type = other DNA
aattttatgctgactcagccccac

SEQ ID NO: 61 - DNA, 22 bp, synthetic construct
  source 1..22: mol_type = other DNA
cagrctgtggtgacycaggagc

SEQ ID NO: 62 - DNA, 20 bp, synthetic construct
  source 1..20: mol_type = other DNA
caggcagggctgactcagcc

SEQ ID NO: 63 - DNA, 20 bp, synthetic construct
  source 1..20: mol_type = other DNA
aggtgtgcacgccgctggtc

SEQ ID NO: 64 - DNA, 23 bp, synthetic construct
  source 1..23: mol_type = other DNA
ggttcggggaagtagtccttgac

SEQ ID NO: 65 - DNA, 24 bp, synthetic construct
  source 1..24: mol_type = other DNA
gtttctcgtagtctgctttgctca

SEQ ID NO: 66 - DNA, 22 bp, synthetic construct
  source 1..22: mol_type = other DNA
gtgctgtccttgctgtcctgct

SEQ ID NO: 67 - DNA, 23 bp, synthetic construct
  source 1..23: mol_type = other DNA
ttggagggtktggtggtctccac

SEQ ID NO: 68 - DNA, 20 bp, synthetic construct
  source 1..20: mol_type = other DNA
ttgacggggctgcyatctgc

SEQ ID NO: 69 - DNA, 21 bp, synthetic construct
  source 1..21: mol_type = other DNA
cacrgctcccgggtagaagtc

SEQ ID NO: 70 - DNA, 41 bp, synthetic construct
  source 1..41: mol_type = other DNA
gttgctacgcgtgtcctgagcsaggtgcagctggtgsagtc

SEQ ID NO: 71 - DNA, 41 bp, synthetic construct
  source 1..41: mol_type = other DNA
gttgctacgcgtgtcctgagccaggtccagcttgtgcagtc

SEQ ID NO: 72 - DNA, 41 bp, synthetic construct
  source 1..41: mol_type = other DNA
gttgctacgcgtgtcctgagccaggttcagctggtgcagtc

SEQ ID NO: 73 - DNA, 43 bp, synthetic construct
  source 1..43: mol_type = other DNA
gttgctacgcgtgtcctgagccaggtccagctggtacagtctg

SEQ ID NO: 74 - DNA, 43 bp, synthetic construct
  source 1..43: mol_type = other DNA
gttgctacgcgtgtcctgagccaggtcaccttgarggagtctg

SEQ ID NO: 75 - DNA, 42 bp, synthetic construct
  source 1..42: mol_type = other DNA
gttgctacgcgtgtcctgagcgaggtgcagctgttggagtct

SEQ ID NO: 76 - DNA, 40 bp, synthetic construct
  source 1..40: mol_type = other DNA
gttgctacgcgtgtcctgagccagstgcagctgcaggagt

SEQ ID NO: 77 - DNA, 42 bp, synthetic construct
  source 1..42: mol_type = other DNA
gttgctacgcgtgtcctgagccaggtgcagctacarcagtgg

SEQ ID NO: 78 - DNA, 42 bp, synthetic construct
  source 1..42: mol_type = other DNA
gttgctacgcgtgtcctgagccaggtacagctgcagcagtca

SEQ ID NO: 79 - DNA, 40 bp, synthetic construct
  source 1..40: mol_type = other DNA
gttgctacgcgtgtcctgagccaggtgcagctggtgcaat

SEQ ID NO: 80 - DNA, 39 bp, synthetic construct
  source 1..39: mol_type = other DNA
gatgggcccttggtgctagctgaggagacggtgaccagg

SEQ ID NO: 81 - DNA, 41 bp, synthetic construct
  source 1..41: mol_type = other DNA
gatgggcccttggtgctagctgaggagacagtgaccagggt

SEQ ID NO: 82 - DNA, 42 bp, synthetic construct
  source 1..42: mol_type = other DNA
gatgggcccttggtgctagctgaagagacggtgaccattgtc

SEQ ID NO: 83 - DNA, 39 bp, synthetic construct
  source 1..39: mol_type = other DNA
gatgggcccttggtgctagctgaggagacggtgaccgtg

SEQ ID NO: 84 - DNA, 43 bp, synthetic construct
  source 1..43: mol_type = other DNA
ggctcccaggtgcacgatgtgacatccagwtgacccagtctcc

SEQ ID NO: 85 - DNA, 47 bp, synthetic construct
  source 1..47: mol_type = other DNA
ggctcccaggtgcacgatgtgatattgtgatgacccagactccactc

SEQ ID NO: 86 - DNA, 45 bp, synthetic construct
  source 1..45: mol_type = other DNA
ggctcccaggtgcacgatgtgaaattgtgttgacrcagtctccag

SEQ ID NO: 87 - DNA, 42 bp, synthetic construct
  source 1..42: mol_type = other DNA
ggctcccaggtgcacgatgtgacatcgtgatgacccagtctc

SEQ ID NO: 88 - DNA, 42 bp, synthetic construct
  source 1..42: mol_type = other DNA
ggctcccaggtgcacgatgtgaaacgacactcacgcagtctc

SEQ ID NO: 89 - DNA, 44 bp, synthetic construct
  source 1..44: mol_type = other DNA
ggctcccaggtgcacgatgtgaaattgtgctgactcagtctcca

SEQ ID NO: 90 - DNA, 37 bp, synthetic construct
  source 1..37: mol_type = other DNA
tgcagccaccgtacgtttgatttccaccttggtccct

SEQ ID NO: 91 - DNA, 37 bp, synthetic construct
  source 1..37: mol_type = other DNA
tgcagccaccgtacgtttgatctccagcttggtccct

SEQ ID NO: 92 - DNA, 37 bp, synthetic construct
  source 1..37: mol_type = other DNA
tgcagccaccgtacgtttgatatccactttggtccca

SEQ ID NO: 93 - DNA, 37 bp, synthetic construct
  source 1..37: mol_type = other DNA
tgcagccaccgtacgtttgatctccaccttggtccct

SEQ ID NO: 94 - DNA, 38 bp, synthetic construct
  source 1..38: mol_type = other DNA
tgcagccaccgtacgtttaatctccagtcgtgtccctt

SEQ ID NO: 95 - DNA, 49 bp, synthetic construct
  source 1..49: mol_type = other DNA
tccttgcttatgggtccggagtggattctcagtctgtgytgacgcagcc

SEQ ID NO: 96 - DNA, 50 bp, synthetic construct
  source 1..50: mol_type = other DNA
tccttgcttatgggtccggagtggattctcagtctgtgctgactcagcca

SEQ ID NO: 97 - DNA, 49 bp, synthetic construct
  source 1..49: mol_type = other DNA
tccttgcttatgggtccggagtggattctcagtctgccctgactcagcc

SEQ ID NO: 98 - DNA, 50 bp, synthetic construct
  source 1..50: mol_type = other DNA
tccttgcttatgggtccggagtggattcttcctatgagctgacwcagcca

SEQ ID NO: 99 - DNA, 50 bp, synthetic construct
  source 1..50: mol_type = other DNA
tccttgcttatgggtccggagtggattcttcttctgagctgactcaggac

SEQ ID NO: 100 - DNA, 49 bp, synthetic construct
  source 1..49: mol_type = other DNA
tccttgcttatgggtccggagtggattctcagsctgtgctgactcagcc

SEQ ID NO: 101 - DNA, 49 bp, synthetic construct
  source 1..49: mol_type = other DNA
tccttgcttatgggtccggagtggattctcagyctgtgctgactcaatc

SEQ ID NO: 102 - DNA, 50 bp, synthetic construct
  source 1..50: mol_type = other DNA
tccttgcttatgggtccggagtggattctaattttatgctgactcagccc

SEQ ID NO: 103 - DNA, 50 bp, synthetic construct
  source 1..50: mol_type = other DNA
tccttgcttatgggtccggagtggattctcagrctgtggtgacycaggag

SEQ ID NO: 104 - DNA, 49 bp, synthetic construct
  source 1..49: mol_type = other DNA
tccttgcttatgggtccggagtggattctcaggcagggctgactcagcc

SEQ ID NO: 105 - DNA, 35 bp, synthetic construct
  source 1..35: mol_type = other DNA
ggccttgggctgacctaggacggtgaccttggtcc

SEQ ID NO: 106 - DNA, 35 bp, synthetic construct
  source 1..35: mol_type = other DNA
ggccttgggctgacctaggacggtcagcttggtcc

SEQ ID NO: 107 - DNA, 35 bp, synthetic construct
  source 1..35: mol_type = other DNA
ggccttgggctgacctaggacggtcaccttggtgc

SEQ ID NO: 108 - DNA, 35 bp, synthetic construct
  source 1..35: mol_type = other DNA
ggccttgggctgacctaggacggtcagctgggtgc

SEQ ID NO: 109 - DNA, 20 bp, synthetic construct
  source 1..20: mol_type = other DNA
gctcccaggtgcacgatgtg

SEQ ID NO: 110 - DNA, 24 bp, synthetic construct
  source 1..24: mol_type = other DNA
gcttatgggtccggagtggattct

SEQ ID NO: 111 - DNA, 20 bp, synthetic construct
  source 1..20: mol_type = other DNA
gatgggcccttggtgctagc

SEQ ID NO: 112 - protein, 8 aa, synthetic construct
GGSISSFS

SEQ ID NO: 113 - protein, 7 aa, synthetic construct
IYYSGST

SEQ ID NO: 114 - protein, 12 aa, synthetic construct
GKGPRSNSPLGV

SEQ ID NO: 115 - protein, 8 aa, synthetic construct
GGSFTRYY

SEQ ID NO: 116 - protein, 7 aa, synthetic construct
ISHNGGP

SEQ ID NO: 117 - protein, 11 aa, synthetic construct
ARETGGDYFDI

SEQ ID NO: 118 - protein, 8 aa, synthetic construct
GGPINNYF

SEQ ID NO: 119 - protein, 7 aa, synthetic construct
IYISGTT

SEQ ID NO: 120 - protein, 9 aa, synthetic construct
ARGADTFDV

SEQ ID NO: 121 - protein, 8 aa, synthetic construct
GGSINSFS

SEQ ID NO: 122 - protein, 7 aa, synthetic construct
IYYSGST

SEQ ID NO: 123 - protein, 10 aa, synthetic construct
GRMLRGRTDS

SEQ ID NO: 124 - protein, 8 aa, synthetic construct
GGSISSYS

SEQ ID NO: 125 - protein, 7 aa, synthetic construct
VYYSGNT

SEQ ID NO: 126 - protein, 11 aa, synthetic construct
VRGAQQRMLAY

SEQ ID NO: 127 - protein, 8 aa, synthetic construct
GFTFSTYD

SEQ ID NO: 128 - protein, 8 aa, synthetic construct
VNGRGDKT

SEQ ID NO: 129 - protein, 12 aa, synthetic construct
VMETPSSAWSGD

SEQ ID NO: 130 - protein, 8 aa, synthetic construct
GGSFSDYY

SEQ ID NO: 131 - protein, 7 aa, synthetic construct
INHSGST

SEQ ID NO: 132 - protein, 26 aa, synthetic construct
ARGRLRGELPAAGPPHAHKPAMYMDV

SEQ ID NO: 133 - protein, 10 aa, synthetic construct
GGSISNSGHY

SEQ ID NO: 134 - protein, 7 aa, synthetic construct
TSSSGYT

SEQ ID NO: 135 - protein, 15 aa, synthetic construct
ARLKNIWGAPGAFDY

SEQ ID NO: 136 - protein, 8 aa, synthetic construct
GYTFTTYA

SEQ ID NO: 137 - protein, 8 aa, synthetic construct
ISPYKVNT

SEQ ID NO: 138 - protein, 19 aa, synthetic construct
ARLQSPPGSFASGSYYFNP

SEQ ID NO: 139 - protein, 8 aa, synthetic construct
GGTFRSYT

SEQ ID NO: 140 - protein, 8 aa, synthetic construct
IIPVFGTT

SEQ ID NO: 141 - protein, 12 aa, synthetic construct
ARDHSTYYYMDV

SEQ ID NO: 142 - protein, 8 aa, synthetic construct
GGTFSSSA

SEQ ID NO: 143 - protein, 8 aa, synthetic construct
IVPIFRTA

SEQ ID NO: 144 - protein, 13 aa, synthetic construct
AGRSGSYRGAFHD

SEQ ID NO: 145 - protein, 8 aa, synthetic construct
GGNFRSYT

SEQ ID NO: 146 - protein, 8 aa, synthetic construct
IIPVFGTT

SEQ ID NO: 147 - protein, 12 aa, synthetic construct
ARDHSTYYYMDV

SEQ ID NO: 148 - protein, 8 aa, synthetic construct
GFSFSSYW

SEQ ID NO: 149 - protein, 8 aa, synthetic construct
IYPGDSET

SEQ ID NO: 150 - protein, 18 aa, synthetic construct
ARFSGIERITLSGDALDM

SEQ ID NO: 151 - protein, 11 aa, synthetic construct
QSLLHTNEYNY

SEQ ID NO: 152 - skipped

SEQ ID NO: 153 - protein, 9 aa, synthetic construct
MQGLQSPFT

SEQ ID NO: 154 - protein, 6 aa, synthetic construct
QYISKY

SEQ ID NO: 155 - skipped

SEQ ID NO: 156 - protein, 9 aa, synthetic construct
QQSYNTPRT

SEQ ID NO: 157 - protein, 6 aa, synthetic construct
QDIRNY

SEQ ID NO: 158 - skipped

SEQ ID NO: 159 - protein, 9 aa, synthetic construct
QHYYTYPRA

SEQ ID NO: 160 - protein, 9 aa, synthetic construct
NSDVGAYKF

SEQ ID NO: 161 - skipped

SEQ ID NO: 162 - protein, 10 aa, synthetic construct
NSYADSYFYV

SEQ ID NO: 163 - protein, 6 aa, synthetic construct
QSISSW

SEQ ID NO: 164 - skipped

SEQ ID NO: 165 - protein, 9 aa, synthetic construct
QQYNSYPWT

SEQ ID NO: 166 - protein, 9 aa, synthetic construct
NSDVGAYKF

SEQ ID NO: 167 - skipped

SEQ ID NO: 168 - protein, 10 aa, synthetic construct
NSYADSYFYV

SEQ ID NO: 169 - protein, 5 aa, synthetic construct
QTIIT

SEQ ID NO: 170 - skipped

SEQ ID NO: 171 - protein, 9 aa, synthetic construct
QQTHTTPVT

SEQ ID NO: 172 - protein, 6 aa, synthetic construct
QDIGNY

SEQ ID NO: 173 - skipped

SEQ ID NO: 174 - protein, 8 aa, synthetic construct
QQYGDLWT

SEQ ID NO: 175 - protein, 6 aa, synthetic construct
QSIGRY

SEQ ID NO: 176 - skipped

SEQ ID NO: 177 - protein, 9 aa, synthetic construct
QQSFNSPPT

SEQ ID NO: 178 - protein, 7 aa, synthetic construct
QSVDNRY

SEQ ID NO: 179 - skipped

SEQ ID NO: 180 - protein, 8 aa, synthetic construct
QQFASTLT

SEQ ID NO: 181 - protein, 6 aa, synthetic construct
QNVSTW

SEQ ID NO: 182 - skipped

SEQ ID NO: 183 - protein, 8 aa, synthetic construct
QQYKSYWT

SEQ ID NO: 184 - protein, 7 aa, synthetic construct
ESVDTRY

SEQ ID NO: 185 - skipped

SEQ ID NO: 186 - protein, 8 aa, synthetic construct
QQFASTLT

SEQ ID NO: 187 - protein, 7 aa, synthetic construct
QSLSSSY

SEQ ID NO: 188 - skipped

SEQ ID NO: 189 - protein, 9 aa, synthetic construct
HQYLSSLWT

SEQ ID NO: 190 - DNA, 429 bp, synthetic construct
  source 1..429: mol_type = other DNA
gatatcgagggtgtggcggcggcgcttacccccgagcggctcctggagtggcaggataaaggaatatttgttatccaaagtgagagtctcaagaaatgcattcaagcaggtaaatcggttctgaccctggagaactgcaagcaagcaaacaagcacatgctgtggaaatgggtttcaaaccatggcctctttaacataggaggcagtggttgcctgggcctgaatttctccgccccagagcagccattaagcttatatgaatgtgactccaccctcgtttccttacggtggcgctgtaacaggaagatgatcacaggcccgctgcagtactctgtccaggtggcgcatgacaacacagtggtggcctcacggaagtatattcataagtggatttcttatgggtcaggtggtggagacatttgtgaatat

SEQ ID NO: 191 - DNA, 429 bp, synthetic construct; identical to SEQ ID NO: 190
  source 1..429: mol_type = other DNA